European Patent Application EP 4 279 510 A1, published November 22, 2023. Title: A Novel Antibody Specific for CD55 and Use Thereof. Applicant: SG medical. The sequence listing filed with the application follows.

SEQUENCE LISTING (48 sequences)

SEQ ID NO: 1 - protein, 17 aa, Artificial Sequence
  HCDR2
GISSSGRYTYYAPAVKG

SEQ ID NO: 2 - protein, 8 aa, Artificial Sequence
  LCDR1
SGGGGSYG

SEQ ID NO: 3 - protein, 10 aa, Artificial Sequence
  LCDR3
GGWDSSTYAI

SEQ ID NO: 4 - protein, 104 aa, Artificial Sequence
  G4-1H_VL
SYELTQPPSVSVSPGQTASITCSGGGGSYGWYQQKPGQSPVTVIYWNDKRPSGIPERFSGSKSGNTATLTISGTQAMDEADYYCGGWDSSTYAIFGGGTKLTVL

SEQ ID NO: 5 - protein, 123 aa, Artificial Sequence
  G4-1H_VH
EVQLVESGGGLVQPGGSLRLSCAASGFTFSDRGMAWVRQAPGKGLEWVSGISSSGRYTYYAPAVKGRATISRDNSKNTLYLQMNSLRAEDTAVYYCAKNAGAGGWHAAYIDAWGQGTTVTVSS

SEQ ID NO: 6 - DNA, 51 bp, Artificial Sequence
  G4-1H VH F primer
cttcctgtcagtaactacaggtgtccactcccaggtgcaactgcagcagtc

SEQ ID NO: 7 - DNA, 39 bp, Artificial Sequence
  G4-1H VH R primer
ccagcgtgaccgtatccagcgcctccaccaagggcccca

SEQ ID NO: 8 - DNA, 17 bp, Artificial Sequence
  G4-1H CH F primer
gcctccaccaagggccc

SEQ ID NO: 9 - DNA, 27 bp, Artificial Sequence
  G4-1H CH R primer
tcccccggcaagtgagcggccgctcac

SEQ ID NO: 10 - DNA, 63 bp, Artificial Sequence
  G4-1H HC F primer
cagaattcactctaaccatggaatggagctgggtctttctcttcttcctgtcagtaactacag

SEQ ID NO: 11 - DNA, 59 bp, Artificial Sequence
  G4-1H VL F primer
ggtctttgtatacatgttgctgtggttgtctggtgttgaaggaagctacgagctgacac

SEQ ID NO: 12 - DNA, 28 bp, Artificial Sequence
  G4-1H VL R primer
caagctcaccgtcttgcggaccgtggcc

SEQ ID NO: 13 - DNA, 20 bp, Artificial Sequence
  G4-1H CK F primer
cggaccgtggccgccccctc

SEQ ID NO: 14 - DNA, 26 bp, Artificial Sequence
  G4-1H CK R primer
cggggcgagtgctagttctagaacta

SEQ ID NO: 15 - DNA, 100 bp, Artificial Sequence
  G4-1H LC F primer
gggaattctagaggatcgaaccctttgcaagcttcggcacgagcagaccagcatgggcatcaagatggagacacattctcaggtctttgtatacatgttg

SEQ ID NO: 16 - DNA, 18 bp, Artificial Sequence
  scFv primer 1
acactttatgcttccggc

SEQ ID NO: 17 - DNA, 20 bp, Artificial Sequence
  scFv primer 2
caaaatcaccggaaccagag

SEQ ID NO: 18 - protein, 104 aa, Artificial Sequence
  EP-1E_VL
SYELTQPPSVSVSPGQTASITCSGGGGSYGWFQQKPGQSPVTVIYWNNKRPSGIPERFSGSKSGNTATLTISGTQAMDEADYYCGGWDSSTYAIFGGGTKLTVL

SEQ ID NO: 19 - protein, 123 aa, Artificial Sequence
  EP-1E_VH
EVQLVESGGGLVQPGGSLRLSCAASGFTFSDRGMAWVRQAPGKGLEWVSGISSSGRYTYYAPAVKGRATISRDNSKNTLYLQMNSLRAEDTAVYYCAKNAVAGGWHAAYIDAWGQGTTVTVSS

SEQ ID NO: 20 - protein, 123 aa, Artificial Sequence
  EP-1F_VH
EVQLAESGGGLVQPGGSLRLSCAASGFTFSDRGMAWVRQAPGKGLEWVSGISSSGRYTYYAPAVKGRATISRDNSKNTLYLQMNSLRAEDTAVYYCAKNAVAGGWHAAYIDAWGQGTTVTVSS

SEQ ID NO: 21 - protein, 123 aa, Artificial Sequence
  EP-9B_VH
EVQLVESGGGLVQPGGSLRLSCAASGFTFSDRGMVWVRQSPGKGLEWVSGISSSGRYTYYAPAVKGRATISRDNSKNTLYLQMNNLRAEDTAVYYCAKNAVAGGWHAAYIDAWGQGTTVTVSS

SEQ ID NO: 22 - protein, 123 aa, Artificial Sequence
  3R-2-1H_VH
EVQLVESGGGLVQPGGSLRLSCVARGFTFSDRGMAWVRQAPGKGLEWVSGISSSGRYTYYAPAVKGRTTISRDNSKNTLYLQMNSLRAEDTAVYYCAKNAVAGGWHAAYIDAWGQGTTVTVSS

SEQ ID NO: 23 - DNA, 46 bp, Artificial Sequence
  VH F primer
cttcctgtcagtaactacaggtgtccactccgaggtccagctggtc

SEQ ID NO: 24 - DNA, 29 bp, Artificial Sequence
  VH R primer
gtgaccgtgtccagcgcctccaccaaggg

SEQ ID NO: 25 - protein, 123 aa, Artificial Sequence
  10H(A)_VH
EVQLVESGGGLVQPGGSLRLSCAASGFTFSDRGMAWVRQAPGKGLEWVSGISSSGRYTYYAPAVKGRATISRDNSKNTLYLQMNSLRAEDTAVYYCAKNAAAGGWHAAYIDAWGQGTTVTVSS

SEQ ID NO: 26 - protein, 123 aa, Artificial Sequence
  10H(I)_VH
EVQLVESGGGLVQPGGSLRLSCAASGFTFSDRGMAWVRQAPGKGLEWVSGISSSGRYTYYAPAVKGRATISRDNSKNTLYLQMNSLRAEDTAVYYCAKNAIAGGWHAAYIDAWGQGTTVTVSS

SEQ ID NO: 27 - protein, 123 aa, Artificial Sequence
  10H(L)_VH
EVQLAESGGGLVQPGGSLRLSCAASGFTFSDRGMAWVRQAPGKGLEWVSGISSSGRYTYYAPAVKGRATISRDNSKNTLYLQMNSLRAEDTAVYYCAKNALAGGWHAAYIDAWGQGTTVTVSS

SEQ ID NO: 28 - protein, 123 aa, Artificial Sequence
  10H(F)_VH
EVQLAESGGGLVQPGGSLRLSCAASGFTFSDRGMAWVRQAPGKGLEWVSGISSSGRYTYYAPAVKGRATISRDNSKNTLYLQMNSLRAEDTAVYYCAKNAFAGGWHAAYIDAWGQGTTVTVSS

SEQ ID NO: 29 - protein, 123 aa, Artificial Sequence
  10H(M)_VH
EVQLAESGGGLVQPGGSLRLSCAASGFTFSDRGMAWVRQAPGKGLEWVSGISSSGRYTYYAPAVKGRATISRDNSKNTLYLQMNSLRAEDTAVYYCAKNAMAGGWHAAYIDAWGQGTTVTVSS

SEQ ID NO: 30 - DNA, 16 bp, Artificial Sequence
  HC1 R primer
gtactactgcgccaag

SEQ ID NO: 31 - DNA, 42 bp, Artificial Sequence
  HC2 F1 primer
gtactactgcgccaagaacgccgcggccggggggtggcacgc

SEQ ID NO: 32 - DNA, 42 bp, Artificial Sequence
  HC2 F2 primer
gtactactgcgccaagaacgccattgccggggggtggcacgc

SEQ ID NO: 33 - DNA, 42 bp, Artificial Sequence
  HC2 F3 primer
gtactactgcgccaagaacgccctggccggggggtggcacgc

SEQ ID NO: 34 - DNA, 42 bp, Artificial Sequence
  HC2 F4 primer
gtactactgcgccaagaacgccatggccggggggtggcacgc

SEQ ID NO: 35 - DNA, 42 bp, Artificial Sequence
  HC2 F5 primer
gtactactgcgccaagaacgcctttgccggggggtggcacgc

SEQ ID NO: 36 - DNA, 33 bp, Artificial Sequence
  CD55-scFv-knob_VL F primer
cagcgcgcactccagctacgagctgacacagcc

SEQ ID NO: 37 - DNA, 61 bp, Artificial Sequence
  CD55-scFv-knob_VL R primer
gaccaagctcaccgtcttgggcggaggcgggagtggtggtggcggtagcggtggaggaggc

SEQ ID NO: 38 - DNA, 45 bp, Artificial Sequence
  CD55-scFv-knob_VH F primer
gtggaggaggcagtggatctggcggctctgaggtccagctggtcg

SEQ ID NO: 39 - DNA, 47 bp, Artificial Sequence
  CD55-scFv-knob_VH R primer
ggcacaaccgtgaccgtgtccagcggcggctcagacaaaactcacac

SEQ ID NO: 40 - DNA, 37 bp, Artificial Sequence
  CD55-scFv-knob_CH F primer
cgtgtccagcggcggctcagacaaaactcacacatgc

SEQ ID NO: 41 - DNA, 33 bp, Artificial Sequence
  CD55-scFv-knob_CH R primer
ctctccctgtccccgggtaaatgactagaacta

SEQ ID NO: 42 - DNA, 45 bp, Artificial Sequence
  CD20-Fab-hole VL-CK F primer
cgcagcgagcgcgcactcccagattgtcctgtctcagtctcctgc

SEQ ID NO: 43 - DNA, 44 bp, Artificial Sequence
  CD20-Fab-hole VL-CK R primer
cggccgccgtgcgagatcttttgatttccagtttagttccgccg

SEQ ID NO: 44 - DNA, 23 bp, Artificial Sequence
  CD20-Fab-hole VH F primer
caagtccaactgcaacaaccggg

SEQ ID NO: 45 - DNA, 50 bp, Artificial Sequence
  CD20-Fab-hole VH R primer
ggaagaccgatgggcccttgaagctagcggcggaaaccgttgtgccagag

SEQ ID NO: 46 - DNA, 15 bp, Artificial Sequence
  CD20-Fab-hole CH F primer
gcaagcttcaagggc

SEQ ID NO: 47 - protein, 477 aa, Artificial Sequence
  CD55-scFv-knob
SYELTQPPSVSVSPGQTASITCSGGGGSYGWYQQKPGQSPVTVIYWNDKRPSGIPERFSGSKSGNTATLTISGTQAMDEADYYCGGWDSSTYAIFGGGTKLTVLGGGGSGGGGSGGGGSGSGGSEVQLVESGGGLVQPGGSLRLSCAASGFTFSDRGMAWVRQAPGKGLEWVSGISSSGRYTYYAPAVKGRATISRDNSKNTLYLQMNSLRAEDTAVYYCAKNAVAGGWHAAYIDAWGQGTTVTVSSGGSDKTHTCPPCPAPELLGGPSVFLFPPKPKDTLMISRTPEVTCVVVDVSHEDPEVKFNWYVDGVEVHNAKTKPREEQYNSTYRVVSVLTVLHQDWLNGKEYKCKVSNKALPAPIEKTISKAKGQPREPQVYTLPPSRDELTKNQVSLWCLVKGFYPSDIAVEWESNGQPENNYKTTPPVLDSDGSFFLYSKLTVDKSRWQQGNVFSCSVMHEALHNHYTQKSLSLSPGK

SEQ ID NO: 48 - protein, 706 aa, Artificial Sequence
  CD20-Fab-hole
QIVLSQSPAILSASPGEKVTMTCRASSSVSYIHWFQQKPGSSPKPWIYATSNLASGVPVRFSGSGSGTSYSLTISRVEAEDAATYYCQQWTSNPPTFGGGTKLEIKRSRTAAAPSVFIFPPSDEQLKSGTASVVCLLNNFYPREAKVQWKVDNALQSGNSQESVTEQDSKDSTYSLSSTLTLSKADYEKHKVYACEVTHQGLSSPVTKSFNRGECGGGGSGGGGSGGGGSGSGGSGGGGSGGGGSGGGGSGSGSSQVQLQQPGAELVKPGASVKMSCKASGYTFTSYNMHWVKQTPGRGLEWIGAIYPGNGDTSYNQKFKGKATLTADKSSSTAYMQLSSLTSEDSAVYYCARSTYYGGDWYFNVWGAGTTVTVSAASFKGPSVFPLAPSSKSTSGGTAALGCLVKDYFPEPVTVSWNSGALTSGVHTFPAVLQSSGLYSLSSVVTVPSSSLGTQTYICNVNHKPSNTKVDKKVEPKSCDKTHTCPPCPAPELLGGPSVFLFPPKPKDTLMISRTPEVTCVVVDVSHEDPEVKFNWYVDGVEVHNAKTKPREEQYNSTYRVVSVLTVLHQDWLNGKEYKCKVSNKALPAPIEKTISKAKGQPREPQVYTLPPSRDELTKNQVSLSCAVKGFYPSDIAVEWESNGQPENNYKTTPPVLDSDGSFFLVSKLTVDKSRWQQGNVFSCSVMHEALHNHYTQKSLSLSPGK